European Patent Application EP 4 530 299 A1, published April 2, 2025. Title: STABLE ANTIBODY PREPARATION. Applicant: REGENECORE BIOTECH CO., LTD. The sequence listing filed with the application follows.

SEQUENCE LISTING (21 sequences)

SEQ ID NO: 1 - protein, 6 aa, synthetic construct
SGDFYC

SEQ ID NO: 2 - protein, 8 aa, synthetic construct
IRSGGRST

SEQ ID NO: 3 - protein, 12 aa, synthetic construct
AVGVDGNCRNYW

SEQ ID NO: 4 - protein, 10 aa, synthetic construct
GNTFSFSTYC

SEQ ID NO: 5 - protein, 7 aa, synthetic construct
TIYDAST

SEQ ID NO: 6 - protein, 15 aa, synthetic construct
AAARYCMFWSHPSYW

SEQ ID NO: 7 - protein, 115 aa, synthetic construct
QVQLVESGGGLVQPGGSLRLSCAASGDFYCMAWFRQAPGKEREAVAAIRSGGRSTYYADSVKGRFTISRDNSKNTLYLQMNSLKAEDTAVYYCAVGVDGNCRNYWGQGTLVTVSS

SEQ ID NO: 8 - protein, 122 aa, synthetic construct
QVQLVESGGGSVQAGGSLRLSCAASGNTFSFSTYCMGWFRQSPGKEREGSLATIYDASTAYAGSVKGRFTISRDNSKNILYLQMNNLRAEDTAVYYCAAARYCMFWSHPSYWGQGTQVTVSS

SEQ ID NO: 9 - protein, 478 aa, synthetic construct
QVQLVESGGGLVQPGGSLRLSCAASGDFYCMAWFRQAPGKEREAVAAIRSGGRSTYYADSVKGRFTISRDNSKNTLYLQMNSLKAEDTAVYYCAVGVDGNCRNYWGQGTLVTVSSESKYGPPCPSCPAPEFLGGPSVFLFPPKPKDTLMISRTPEVTCVVVDVSQEDPEVQFNWYVDGVEVHNAKTKPREEQFNSTYRVVSVLTVLHQDWLNGKEYKCKVSNKGLPSSIEKTISKAKGQPREPQVYTLPPSQEEMTKNQVSLTCLVKGFYPSDIAVEWESNGQPENNYKTTPPVLDSDGSFFLYSRLTVDKSRWQEGNVFSCSVMHEALHNHYTQKSLSLSLGKESKYGPPCPSCPQVQLVESGGGSVQAGGSLRLSCAASGNTFSFSTYCMGWFRQSPGKEREGSLATIYDASTAYAGSVKGRFTISRDNSKNILYLQMNNLRAEDTAVYYCAAARYCMFWSHPSYWGQGTQVTVSS

SEQ ID NO: 10 - protein, 478 aa, synthetic construct
QVQLVESGGGLVQPGGSLRLSCAASGDFYCMAWFRQAPGKEREAVAAIRSGGRSTYYADSVKGRFTISRDNSKNTLYLQMNSLKAEDTAVYYCAVGVDGNCRNYWGQGTLVTVSSESKYGPPCPPCPAPEFLGGPSVFLFPPKPKDTLMISRTPEVTCVVVDVSQEDPEVQFNWYVDGVEVHNAKTKPREEQFNSTYRVVSVLTVLHQDWLNGKEYKCKVSNKGLPSSIEKTISKAKGQPREPQVYTLPPSQEEMTKNQVSLTCLVKGFYPSDIAVEWESNGQPENNYKTTPPVLDSDGSFFLYSRLTVDKSRWQEGNVFSCSVMHEALHNHYTQKSLSLSLGKESKYGPPCPPCPQVQLVESGGGSVQAGGSLRLSCAASGNTFSFSTYCMGWFRQSPGKEREGSLATIYDASTAYAGSVKGRFTISRDNSKNILYLQMNNLRAEDTAVYYCAAARYCMFWSHPSYWGQGTQVTVSS

SEQ ID NO: 11 - DNA, 1434 bp, synthetic construct
  source 1..1434: mol_type = other DNA
caagtgcaacttgtggaatcaggaggaggatcagtgcaagcaggaggatcacttagactttcatgcgcagcatcaggagatttctattgtatggcatggtttagacaagcacctggaaaggagagggaaggagtggcaacaatcagatcaggaggaagatcaacatactacgcagattcagtgaaaggaagatttacaatctcaaaggacaatgcaaaggacaccctttaccttcaaatgaactcacttaaacctgaagatacagcaatgtactactgcgcagtgggagtggatggaaactgcagaaactactggggccaggggacacaagtgacagtgtcatcagagagcaagtacggccctccttgccccagctgccccgcccccgagtttctgggaggccccagcgtgtttctgtttcctcccaagcccaaagacacactgatgatcagcagaacccccgaggtgacatgcgtggtggtcgacgtgagccaagaagatcccgaggtgcagttcaactggtatgtggacggcgtggaggtgcacaacgccaagaccaagcctagggaggagcaattcaacagcacctacagagtggtgagcgtgctgaccgtgctgcaccaagactggctgaacggcaaggagtataagtgtaaggtgagcaacaagggcctccccagcagcatcgagaagaccatctccaaggccaagggccagcctagggagcctcaagtgtacacactgccccccagccaagaggagatgaccaaaaaccaagtgtctctgacatgcctcgtgaagggcttctatcccagcgacatcgccgtggagtgggagagcaatggccagcccgagaataactacaagaccaccccccccgtgctcgactccgatggcagcttctttctgtactctaggctgaccgtggacaagtctaggtggcaagagggaaacgtgttcagctgttccgtgatgcacgaggctctgcacaaccactacacccagaagagcctctctctgtctctgggaaaggagagcaagtacggccctccttgccccagctgcccccaagtgcagctggtggagagtgggggcggtagcgtacaagcgggcggcagcctgagactgagctgcgccgccagcggcaacaccttcagcttcagcacctactgcatgggctggttcagacagagccccggcaaggagagagagggcagcctggccaccatctacgacgccagcaccgcctacgccggcagcgtgaagggcagattcaccatcagcagagacaacagcaagaacatcctgtacctgcagatgaacaacctgagagccgaggacaccgccgtgtactactgcgccgccgccagatactgcatgttctggagccaccccagctactggggccagggcacccaggtgaccgtgagcagc

SEQ ID NO: 12 - DNA, 1434 bp, synthetic construct
  source 1..1434: mol_type = other DNA
caagtgcagctggtggagagtgggggcggtctggtacaaccgggcggcagcctgagactgagctgcgccgccagcggcgacttctactgcatggcctggttcagacaggcccccggcaaggagagagaggccgtggccgccatcagaagcggcggcagaagcacctactacgccgacagcgtgaagggcagattcaccatcagcagagacaacagcaagaacaccctgtacctgcagatgaacagcctgaaggccgaggacaccgccgtgtactactgcgccgtgggcgtggacggcaactgcagaaactactggggccagggcaccctggtgaccgtgagcagcgagagcaagtacggccctccttgccccccttgccccgcccccgagtttctgggaggccccagcgtgtttctgtttcctcccaagcccaaagacacactgatgatcagcagaacccccgaggtgacatgcgtggtggtcgacgtgagccaagaagatcccgaggtgcagttcaactggtatgtggacggcgtggaggtgcacaacgccaagaccaagcctagggaggagcaattcaacagcacctacagagtggtgagcgtgctgaccgtgctgcaccaagactggctgaacggcaaggagtataagtgtaaggtgagcaacaagggcctccccagcagcatcgagaagaccatctccaaggccaagggccagcctagggagcctcaagtgtacacactgccccccagccaagaggagatgaccaaaaaccaagtgtctctgacatgcctcgtgaagggcttctatcccagcgacatcgccgtggagtgggagagcaatggccagcccgagaataactacaagaccaccccccccgtgctcgactccgatggcagcttctttctgtactctaggctgaccgtggacaagtctaggtggcaagagggaaacgtgttcagctgttccgtgatgcacgaggctctgcacaaccactacacccagaagagcctctctctgtctctgggaaaggagagcaagtacggccctccttgccccccttgcccccaagtgcagctggtggagagtgggggcggtagcgtacaagcgggcggcagcctgagactgagctgcgccgccagcggcaacaccttcagcttcagcacctactgcatgggctggttcagacagagccccggcaaggagagagagggcagcctggccaccatctacgacgccagcaccgcctacgccggcagcgtgaagggcagattcaccatcagcagagacaacagcaagaacatcctgtacctgcagatgaacaacctgagagccgaggacaccgccgtgtactactgcgccgccgccagatactgcatgttctggagccaccccagctactggggccagggcacccaggtgaccgtgagcagc

SEQ ID NO: 13 - protein, 241 aa, synthetic construct
ESKYGPPCPPCPAPEFLGGPSVFLFPPKPKDTLMISRTPEVTCVVVDVSQEDPEVQFNWYVDGVEVHNAKTKPREEQFNSTYRVVSVLTVLHQDWLNGKEYKCKVSNKGLPSSIEKTISKAKGQPREPQVYTLPPSQEEMTKNQVSLTCLVKGFYPSDIAVEWESNGQPENNYKTTPPVLDSDGSFFLYSRLTVDKSRWQEGNVFSCSVMHEALHNHYTQKSLSLSLGKESKYGPPCPPCP

SEQ ID NO: 14 - protein, 24 aa, synthetic construct
QVQLVESGGGLVQPGGSLRLSCAA

SEQ ID NO: 15 - protein, 17 aa, synthetic construct
MAWFRQAPGKEREAVAA

SEQ ID NO: 16 - protein, 38 aa, synthetic construct
YYADSVKGRFTISRDNSKNTLYLQMNSLKAEDTAVYYC

SEQ ID NO: 17 - protein, 10 aa, synthetic construct
GQGTLVTVSS

SEQ ID NO: 18 - protein, 25 aa, synthetic construct
QVQLVESGGGSVQAGGSLRLSCAAS

SEQ ID NO: 19 - protein, 17 aa, synthetic construct
MGWFRQSPGKEREGSLA

SEQ ID NO: 20 - protein, 38 aa, synthetic construct
AYAGSVKGRFTISRDNSKNILYLQMNNLRAEDTAVYYC

SEQ ID NO: 21 - protein, 10 aa, synthetic construct
GQGTQVTVSS